European Patent Specification EP 4 179 320 B1, published July 31, 2024. Title: System for study of tau aggregation. Applicant: WisTa Laboratories Ltd. The sequence listing filed with the application follows.

SEQUENCE LISTING (18 sequences)

SEQ ID NO: 1 - protein, 441 aa, Homo sapiens
MAEPRQEFEVMEDHAGTYGLGDRKDQGGYTMHQDQEGDTDAGLKESPLQTPTEDGSEEPGSETSDAKSTPTAEDVTAPLVDEGAPGKQAAAQPHTEIPEGTTAEEAGIGDTPSLEDEAAGHVTQARMVSKSKDGTGSDDKKAKGADGKTKIATPRGAAPPGQKGQANATRIPAKTPPAPKTPPSSGEPPKSGDRSGYSSPGSPGTPGSRSRTPSLPTPPTREPKKVAVVRTPPKSPSSAKSRLQTAPVPMPDLKNVKSKIGSTENLKHQPGGGKVQIINKKLDLSNVQSKCGSKDNIKHVPGGGSVQIVYKPVDLSKVTSKCGSLGNIHHKPGGGQVEVKSEKLDFKDRVQSKIGSLDNITHVPGGGNKKIETHKLTFRENAKAKTDHGAEIVYKSPVVSGDTSPRHLSNVSSTGSIDMVDSPQLATLADEVSASLAKQGL

SEQ ID NO: 2 - protein, 758 aa, Homo sapiens
MAEPRQEFEVMEDHAGTYGLGDRKDQGGYTMHQDQEGDTDAGLKESPLQTPTEDGSEEPGSETSDAKSTPTAEDVTAPLVDEGAPGKQAAAQPHTEIPEGTTAEEAGIGDTPSLEDEAAGHVTQEPESGKVVQEGFLREPGPPGLSHQLMSGMPGAPLLPEGPREATRQPSGTGPEDTEGGRHAPELLKHQLLGDLHQEGPPLKGAGGKERPGSKEEVDEDRDVDESSPQDSPPSKASPAQDGRPPQTAAREATSIPGFPAEGAIPLPVDFLSKVSTEIPASEPDGPSVGRAKGQDAPLEFTFHVEITPNVQKEQAHSEEHLGRAAFPGAPGEGPEARGPSLGEDTKEADLPEPSEKQPAAAPRGKPVSRVPQLKARMVSKSKDGTGSDDKKAKTSTRSSAKTLKNRPCLSPKHPTPGSSDPLIQPSSPAVCPEPPSSPKYVSSVTSRTGSSGAKEMKLKGADGKTKIATPRGAAPPGQKGQANATRIPAKTPPAPKTPPSSGEPPKSGDRSGYSSPGSPGTPGSRSRTPSLPTPPTREPKKVAVVRTPPKSPSSAKSRLQTAPVPMPDLKNVKSKIGSTENLKHQPGGGKVQIINKKLDLSNVQSKCGSKDNIKHVPGGGSVQIVYKPVDLSKVTSKCGSLGNIHHKPGGGQVEVKSEKLDFKDRVQSKIGSLDNITHVPGGGNKKIETHKLTFRENAKAKTDHGAEIVYKSPVVSGDTSPRHLSNVSSTGSIDMVDSPQLATLADEVSASLAKQGL

SEQ ID NO: 3 - protein, 97 aa, Homo sapiens
DNIKHVPGGGSVQIVYKPVDLSKVTSKCGSLGNIHHKPGGGQVEVKSEKLDFKDRVQSKIGSLDNITHVPGGGNKKIETHKLTFRENAKAKTDHGAE

SEQ ID NO: 4 - protein, 95 aa, Homo sapiens
IKHVPGGGSVQIVYKPVDLSKVTSKCGSLGNIHHKPGGGQVEVKSEKLDFKDRVQSKIGSLDNITHVPGGGNKKIETHKLTFRENAKAKTDHGAE

SEQ ID NO: 5 - protein, 94 aa, Homo sapiens
IKHVPGGGSVQIVYKPVDLSKVTSKCGSLGNIHHKPGGGQVEVKSEKLDFKDRVQSKIGSLDNITHVPGGGNKKIETHKLTFRENAKAKTDHGA

SEQ ID NO: 6 - protein, 73 aa, Homo sapiens
VQIVYKPVDLSKVTSKCGSLGNIHHKPGGGQVEVKSEKLDFKDRVQSKIGSLDNITHVPGGGNKKIETHKLTF

SEQ ID NO: 7 - protein, 71 aa, Homo sapiens
IVYKPVDLSKVTSKCGSLGNIHHKPGGGQVEVKSEKLDFKDRVQSKIGSLDNITHVPGGGNKKIETHKLTF

SEQ ID NO: 8 - protein, 13 aa, artificial sequence
  S1D12 epitope
VEVKSEKLDFKDR

SEQ ID NO: 9 - protein, 5 aa, artificial sequence
  VHCDR1 S1D12
NNAVG

SEQ ID NO: 10 - protein, 16 aa, artificial sequence
  VHCDR2 S1D12
GCSSDGTCYYNSALKS

SEQ ID NO: 11 - protein, 16 aa, artificial sequence
  VHCDR3 S1D12
GHYSIYGYDYLGTIDY

SEQ ID NO: 12 - protein, 14 aa, artificial sequence
  VLCDR1 S1D12
SGSSSNVGGGNSVG

SEQ ID NO: 13 - protein, 7 aa, artificial sequence
  VLCDR2 S1D12
DTNSRPS

SEQ ID NO: 14 - protein, 11 aa, artificial sequence
  VLCDR3 S1D12
VTGDSTTHDDL

SEQ ID NO: 15 - protein, 123 aa, artificial sequence
  VH Domain S1D12
QVQLQESGPSLVKPSQTLSLTCTVSGFSLNNNAVGWVRQAPGKVPESLVGCSSDGTCYYNSALKSRLDITRDTSKNQISLSLSSVTTDDAAVYYCTRGHYSIYGYDYLGTIDYWGPGLLVTVS

SEQ ID NO: 16 - protein, 112 aa, artificial sequence
  VL Domain S1D12
QAVLTQPSSVSGSLGQRVSITCSGSSSNVGGGNSVGWYQHLPGSGLKTIIYDTNSRPSGVPDRFSGSRSGNTATLTINSLQAEDEGDYYCVTGDSTTHDDLVGSGTRLTVLG

SEQ ID NO: 17 - protein, 454 aa, artificial sequence
  S1D12 Heavy Chain
QVQLQESGPSLVKPSQTLSLTCTVSGFSLNNNAVGWVRQAPGKVPESLVGCSSDGTCYYNSALKSRLDITRDTSKNQISLSLSSVTTDDAAVYYCTRGHYSIYGYDYLGTIDYWGPGLLVTVSSAKTTAPSVYPLAPVCGDTTGSSVTLGCLVKGYFPEPVTLTWNSGSLSSGVHTFPAVLQSDLYTLSSSVTVTSSTWPSQSITCNVAHPASSTKVDKKIEPRGPTIKPCPPCKCPAPNLLGGPSVFIFPPKIKDVLMISLSPIVTCVVVDVSEDDPDVQISWFVNNVEVHTAQTQTHREDYNSTLRVVSALPIQHQDWMSGKEFKCKVNNKDLPAPIERTISKPKGSVRAPQVYVLPPPEEEMTKKQVTLTCMVTDFMPEDIYVEWTNNGKTELNYKNTEPVLDSDGSYFMYSKLRVEKKNWVERNSYSCSVVHEGLHNHHTTKSFSRTPGK

SEQ ID NO: 18 - protein, 218 aa, artificial sequence
  S1D12 Light Chain
QAVLTQPSSVSGSLGQRVSITCSGSSSNVGGGNSVGWYQHLPGSGLKTIIYDTNSRPSGVPDRFSGSRSGNTATLTINSLQAEDEGDYYCVTGDSTTHDDLVGSGTRLTVLGGQPKSSPSVTLFPPSSEELETNKATLVCTITDFYPGVVTVDWKVDGTPVTQGMETTQPSKQSNNKYMASSYLTLTARAWERHSSYSCQVTHEGHTVEKSLSRADCS